European Patent Application EP 4 772 185 A1, published July 8, 2026. Title: Compositions for skin wound or scar treatment comprising mesenchymal stem cell spheroids. Applicant: 주식회사 셀인셀즈. The sequence listing filed with the application follows.

SEQUENCE LISTING (30 sequences)

SEQ ID NO: 1 - DNA, 19 bp, synthetic construct
  source 1..19: mol_type = other DNA
atggggaaggtgaaggtcg

SEQ ID NO: 2 - DNA, 20 bp, synthetic construct
  source 1..20: mol_type = other DNA
taaaagcagccctggtgacc

SEQ ID NO: 3 - DNA, 21 bp, synthetic construct
  source 1..21: mol_type = other DNA
tacagggcggccacaagtttt

SEQ ID NO: 4 - DNA, 21 bp, synthetic construct
  source 1..21: mol_type = other DNA
atggagagcaaagccctgctc

SEQ ID NO: 5 - DNA, 20 bp, synthetic construct
  source 1..20: mol_type = other DNA
catcagtgtgaatggggatg

SEQ ID NO: 6 - DNA, 20 bp, synthetic construct
  source 1..20: mol_type = other DNA
gtggaagtgacgcctttcat

SEQ ID NO: 7 - DNA, 20 bp, synthetic construct
  source 1..20: mol_type = other DNA
gaccactcccactcctttga

SEQ ID NO: 8 - DNA, 20 bp, synthetic construct
  source 1..20: mol_type = other DNA
cgacattcaattgccatgag

SEQ ID NO: 9 - DNA, 25 bp, synthetic construct
  source 1..25: mol_type = other DNA
tatgaaaaaccaagtagcaaggttc

SEQ ID NO: 10 - DNA, 25 bp, synthetic construct
  source 1..25: mol_type = other DNA
gtaatctgactctgtccttgtggat

SEQ ID NO: 11 - DNA, 20 bp, synthetic construct
  source 1..20: mol_type = other DNA
gtgcagagtccagcaaaggt

SEQ ID NO: 12 - DNA, 20 bp, synthetic construct
  source 1..20: mol_type = other DNA
ctagccaactcgtcacagtc

SEQ ID NO: 13 - DNA, 24 bp, synthetic construct
  source 1..24: mol_type = other DNA
ttcagtggcctaccaagtggcata

SEQ ID NO: 14 - DNA, 24 bp, synthetic construct
  source 1..24: mol_type = other DNA
agcctgggttacagattccaccaa

SEQ ID NO: 15 - DNA, 20 bp, synthetic construct
  source 1..20: mol_type = other DNA
tttcccaggtcaagatggtc

SEQ ID NO: 16 - DNA, 20 bp, synthetic construct
  source 1..20: mol_type = other DNA
ctgcagcacctgtctcacca

SEQ ID NO: 17 - DNA, 24 bp, synthetic construct
  source 1..24: mol_type = other DNA
atgacccaaggactggaatcttta

SEQ ID NO: 18 - DNA, 23 bp, synthetic construct
  source 1..23: mol_type = other DNA
ctgagaaagaggagtggacatac

SEQ ID NO: 19 - DNA, 20 bp, synthetic construct
  source 1..20: mol_type = other DNA
ccactcctccacctttgacg

SEQ ID NO: 20 - DNA, 20 bp, synthetic construct
  source 1..20: mol_type = other DNA
ccaccaccctgttgctgtag

SEQ ID NO: 21 - DNA, 22 bp, synthetic construct
  source 1..22: mol_type = other DNA
tgcagattatgcggatcaaacc

SEQ ID NO: 22 - DNA, 25 bp, synthetic construct
  source 1..25: mol_type = other DNA
tgcattcacatttgttgtgctgtag

SEQ ID NO: 23 - DNA, 20 bp, synthetic construct
  source 1..20: mol_type = other DNA
tgtggagacaggggctttta

SEQ ID NO: 24 - DNA, 20 bp, synthetic construct
  source 1..20: mol_type = other DNA
cctgcactccctctacttgc

SEQ ID NO: 25 - DNA, 21 bp, synthetic construct
  source 1..21: mol_type = other DNA
tcacgagcatgacatgactcc

SEQ ID NO: 26 - DNA, 21 bp, synthetic construct
  source 1..21: mol_type = other DNA
agcttacttgcatctggttcc

SEQ ID NO: 27 - DNA, 20 bp, synthetic construct
  source 1..20: mol_type = other DNA
tcaaaggagtgtgtgcgaac

SEQ ID NO: 28 - DNA, 19 bp, synthetic construct
  source 1..19: mol_type = other DNA
cagggccacataccaactg

SEQ ID NO: 29 - DNA, 20 bp, synthetic construct
  source 1..20: mol_type = other DNA
tccatgccactaagcatgtg

SEQ ID NO: 30 - DNA, 22 bp, synthetic construct
  source 1..22: mol_type = other DNA
cgtaaatgaccgtcctggtctt